European Patent Specification EP 3 823 654 B1, published February 14, 2024. Title: METHODS FOR TREATMENT OF CANCER USING CHIKUNGUNYA-VSV CHIMERIC VIRUS. Applicant: YALE UNIVERSITY VAN DEN POL, ANTHONY N. The sequence listing filed with the application follows.

SEQUENCE LISTING (11 sequences)

SEQ ID NO: 1 - protein, 1248 aa, Chikungunya virus
MEFIPTQTFYNRRYQPRPWTPRPTIQVIRPRPRPQRQAGQLAQLISAVNKLTMRAVPQQKPRRNRKNKKQKQKQQAPQNNTNQKKQPPKKKPAQKKKKPGRRERMCMKIENDCIFEVKHEGKVTGYACLVGDKVMKPAHVKGTIDNADLAKLAFKRSSKYDLECAQIPVHMKSDASKFTHEKPEGYYNWHHGAVQYSGGRFTIPTGAGKPGDSGRPIFDNKGRVVAIVLGGANEGARTALSVVTWNKDIVTKITPEGAEEWSLAIPVMCLLANTTFPCSQPPCIPCCYEKEPEETLRMLEDNVMRPGYYQLLQASLTCSPHRQRRSTKDNFNVYKATRPYLAHCPDCGEGHSCHSPVALERIRNEATDGTLKIQVSLQIGIGTDDSHDWTKLRYMDNHIPADAGRAGLFVRTSAPCTITGTMGHFILARCPKGETLTVGFTDSRKISHSCTHPFHHDPPVIGREKFHSRPQHGKELPCSTYVQSNAATAEEIEVHMPPDTPDRTLLSQQSGNVKITVNGRTVRYKCNCGGSNEGLITTDKVINNCKVDQCHAAVTNHKKWQYNSPLVPRNAELGDRKGKIHIPFPLANVTCMVPKARNPTVTYGKNQVIMLLYPDHPTLLSYRSMGEEPNYQEEWVTHKKEVVLTVPTEGLEVTWGNNEPYKYWPQLSANGTAHGHPHEIILYYYELYPTMTVVVVSVASFILLSMVGMAVGMCMCARRRCITPYELTPGATVPFLLSLICCIRTAKAATYQEAAVYLWNEQQPLFWLQALIPLAALIVLCNCLRLLPCCCKTLAFLAVMSIGAHTVSAYEHVTVIPNTVGVPYKTLVNRPGYSPMVLEMELLSVTLEPTLSLDYITCEYKTVIPSPYVKCCGTAECKDKNLPDYSCKVFTGVYPFMWGGAYCFCDAENTQLSEAHVEKSESCKTEFASAYRAHTASASAKLRVLYQGNNITVTAYANGDHAVTVKDAKFIVGPMSSAWTPFDNKIVVYKGDVYNMDYPPFGAGRPGQFGDIQSRTPESKDVYANTQLVLQRPAAGTVHVPYSQAPSGFKYWLKERGASLQHTAPFGCQIATNPVRAMNCAVGNMPISIDIPDAAFTRVVDAPSLTDMSCEVPACTHSSDFGGVAIIKYAVSKKGKCAVHSMTNAVTIREAEIEVEGNSQLQISFSTALASAEFRVQVCSTQVHCAAECHPPKDHIVNYPASHTTLGVQDISATAMSWVQKITGGVGLVVAVAALILIVVLCVSFSRH

SEQ ID NO: 2 - protein, 1248 aa, Chikungunya virus
MEFIPTQTFYNRRYQPRPWTPRPTIQVIRPRPRPQRQAGQLAQLISAVNKLTMRAVPQQKPRKNRKNKKQKQKQQAPQNNTNQKKQPPKKKPAQKKKKPGRRERMCMKIENDCIFEVKHEGKVTGYACLVGDKVMKPAHVKGTIDNADLAKLAFKRSSKYDLECAQIPVHMKSDASKFTHEKPEGYYNWHHGAVQYSGGRFTIPTGAGKPGDSGRPIFDNKGRVVAIVLGGANEGARTALSVVTWNKDIVTKITPEGAEEWSLAIPVMCLLANTTFPCSQPPCIPCCYEKEPEETLRMLEDNVMRPGYYQLLQASLTCSPHRQRRSTKDNFNVYKATRPYLAHCPDCGEGHSCHSPVALERIRNEATDGTLKIQVSLQIGIGTDDSHDWTKLRYMDNHIPADAGRAGLFVRTSAPCTITGTMGHFILARCPKGETLTVGFTDSRKISHSCTHPFHHDPPVIGREKFHSRPQHGKELPCSTYVQSNAATAEEIEVHMPPDTPDRTLLSQQSGNVKITVNSQTVRYKCNCGGSNEGLITTDKVINNCKVDQCHAAVTNHKKWQYNSPLVPRNAELGDRKGKIHIPFPLANVTCMVPKARNPTVTYGKNQVIMLLYPDHPTLLSYRSMGEEPNYQEEWVTHKKEVVLTVPTEGLEVTWGNNEPYKYWPQLSANGTAHGHPHEIILYYYELYPTMTVVVVSVASFILLSMVGMAVGMCMCARRRCITPYELTPGATVPFLLSLICCIRTAKAATYQEAAVYLWNEQQPLFWLQALIPLAALIVLCNCLRLLPCCCKTLAFLAVMSIGAHTVSAYEHVTVIPNTVGVPYKTLVNRPGYSPMVLEMELLSVTLEPTLSLDYITCEYKTVIPSPYVKCCGTAECKDKNLPDYSCKVFTGVYPFMWGGAYCFCDAENTQLSEAHVEKSESCKTEFASAYRAHTASASAKLRVLYQGNNITVTAYANGDHAVTVKDAKFIVGPMSSAWTPFDNKIVVYKGDVYNMDYPPFGAGRPGQFGDIQSRTPESKDVYANTQLVLQRPAAGTVHVPYSQAPSGFKYWLKERGASLQHTAPFGCQIATNPVRAMNCAVGNMPISIDIPDAAFTRVVDAPSLTDMSCEVPACTHSSDFGGVAIIKYAVSKKGKCAVHSMTNAVTIREAEIEVEGNSQLQISFSTALASAEFRVQVCSTQVHCAAECHPPKDHIVNYPASHTTLGVQDISATAMSWVQKITGGVGLVVAVAALILIVVLCVSFSRH

SEQ ID NO: 3 - protein, 261 aa, Artificial Sequence
  synthetic polypeptide - Q8JUX5, capsid protein
MEFIPTQTFYNRRYQPRPWTPRPTIQVIRPRPRPQRQAGQLAQLISAVNKLTMRAVPQQKPRRNRKNKKQKQKQQAPQNNTNQKKQPPKKKPAQKKKKPGRRERMCMKIENDCIFEVKHEGKVTGYACLVGDKVMKPAHVKGTIDNADLAKLAFKRSSKYDLECAQIPVHMKSDASKFTHEKPEGYYNWHHGAVQYSGGRFTIPTGAGKPGDSGRPIFDNKGRVVAIVLGGANEGARTALSVVTWNKDIVTKITPEGAEEW

SEQ ID NO: 4 - protein, 261 aa, Artificial Sequence
  synthetic polypeptide - NP_690589.2  - capsid protein
MEFIPTQTFYNRRYQPRPWTPRPTIQVIRPRPRPQRQAGQLAQLISAVNKLTMRAVPQQKPRKNRKNKKQKQKQQAPQNNTNQKKQPPKKKPAQKKKKPGRRERMCMKIENDCIFEVKHEGKVTGYACLVGDKVMKPAHVKGTIDNADLAKLAFKRSSKYDLECAQIPVHMKSDASKFTHEKPEGYYNWHHGAVQYSGGRFTIPTGAGKPGDSGRPIFDNKGRVVAIVLGGANEGARTALSVVTWNKDIVTKITPEGAEEW

SEQ ID NO: 5 - protein, 64 aa, Artificial Sequence
  synthetic polypeptide - Q8JUX5 and NP_690589.2 -  Assembly protein E3
SLAIPVMCLLANTTFPCSQPPCIPCCYEKEPEETLRMLEDNVMRPGYYQLLQASLTCSPHRQRR

SEQ ID NO: 6 - protein, 423 aa, Artificial Sequence
  synthetic polypeptide - Q8JUX5 - Spike glycoprotein E2
STKDNFNVYKATRPYLAHCPDCGEGHSCHSPVALERIRNEATDGTLKIQVSLQIGIGTDDSHDWTKLRYMDNHIPADAGRAGLFVRTSAPCTITGTMGHFILARCPKGETLTVGFTDSRKISHSCTHPFHHDPPVIGREKFHSRPQHGKELPCSTYVQSNAATAEEIEVHMPPDTPDRTLLSQQSGNVKITVNGRTVRYKCNCGGSNEGLITTDKVINNCKVDQCHAAVTNHKKWQYNSPLVPRNAELGDRKGKIHIPFPLANVTCMVPKARNPTVTYGKNQVIMLLYPDHPTLLSYRSMGEEPNYQEEWVTHKKEVVLTVPTEGLEVTWGNNEPYKYWPQLSANGTAHGHPHEIILYYYELYPTMTVVVVSVASFILLSMVGMAVGMCMCARRRCITPYELTPGATVPFLLSLICCIRTAKA

SEQ ID NO: 7 - protein, 423 aa, Artificial Sequence
  synthetic polypeptide - NP_690589.2 - Spike glycoprotein E2
STKDNFNVYKATRPYLAHCPDCGEGHSCHSPVALERIRNEATDGTLKIQVSLQIGIGTDDSHDWTKLRYMDNHIPADAGRAGLFVRTSAPCTITGTMGHFILARCPKGETLTVGFTDSRKISHSCTHPFHHDPPVIGREKFHSRPQHGKELPCSTYVQSNAATAEEIEVHMPPDTPDRTLLSQQSGNVKITVNSQTVRYKCNCGGSNEGLITTDKVINNCKVDQCHAAVTNHKKWQYNSPLVPRNAELGDRKGKIHIPFPLANVTCMVPKARNPTVTYGKNQVIMLLYPDHPTLLSYRSMGEEPNYQEEWVTHKKEVVLTVPTEGLEVTWGNNEPYKYWPQLSANGTAHGHPHEIILYYYELYPTMTVVVVSVASFILLSMVGMAVGMCMCARRRCITPYELTPGATVPFLLSLICCIRTAKA

SEQ ID NO: 8 - protein, 61 aa, Artificial Sequence
  synthetic polypeptide - Q8JUX5 and NP_690589.2 - 6K protein
ATYQEAAVYLWNEQQPLFWLQALIPLAALIVLCNCLRLLPCCCKTLAFLAVMSIGAHTVSA

SEQ ID NO: 9 - protein, 439 aa, Artificial Sequence
  synthetic polypeptide - Q8JUX5 and NP_690589.2 - Spike glycoprotein E1
YEHVTVIPNTVGVPYKTLVNRPGYSPMVLEMELLSVTLEPTLSLDYITCEYKTVIPSPYVKCCGTAECKDKNLPDYSCKVFTGVYPFMWGGAYCFCDAENTQLSEAHVEKSESCKTEFASAYRAHTASASAKLRVLYQGNNITVTAYANGDHAVTVKDAKFIVGPMSSAWTPFDNKIVVYKGDVYNMDYPPFGAGRPGQFGDIQSRTPESKDVYANTQLVLQRPAAGTVHVPYSQAPSGFKYWLKERGASLQHTAPFGCQIATNPVRAMNCAVGNMPISIDIPDAAFTRVVDAPSLTDMSCEVPACTHSSDFGGVAIIKYAVSKKGKCAVHSMTNAVTIREAEIEVEGNSQLQISFSTALASAEFRVQVCSTQVHCAAECHPPKDHIVNYPASHTTLGVQDISATAMSWVQKITGGVGLVVAVAALILIVVLCVSFSRH

SEQ ID NO: 10 - protein, 987 aa, Artificial Sequence
  synthetic polypeptide - Q8JUX5 - E3-E2-6K-E1
SLAIPVMCLLANTTFPCSQPPCIPCCYEKEPEETLRMLEDNVMRPGYYQLLQASLTCSPHRQRRSTKDNFNVYKATRPYLAHCPDCGEGHSCHSPVALERIRNEATDGTLKIQVSLQIGIGTDDSHDWTKLRYMDNHIPADAGRAGLFVRTSAPCTITGTMGHFILARCPKGETLTVGFTDSRKISHSCTHPFHHDPPVIGREKFHSRPQHGKELPCSTYVQSNAATAEEIEVHMPPDTPDRTLLSQQSGNVKITVNGRTVRYKCNCGGSNEGLITTDKVINNCKVDQCHAAVTNHKKWQYNSPLVPRNAELGDRKGKIHIPFPLANVTCMVPKARNPTVTYGKNQVIMLLYPDHPTLLSYRSMGEEPNYQEEWVTHKKEVVLTVPTEGLEVTWGNNEPYKYWPQLSANGTAHGHPHEIILYYYELYPTMTVVVVSVASFILLSMVGMAVGMCMCARRRCITPYELTPGATVPFLLSLICCIRTAKAATYQEAAVYLWNEQQPLFWLQALIPLAALIVLCNCLRLLPCCCKTLAFLAVMSIGAHTVSAYEHVTVIPNTVGVPYKTLVNRPGYSPMVLEMELLSVTLEPTLSLDYITCEYKTVIPSPYVKCCGTAECKDKNLPDYSCKVFTGVYPFMWGGAYCFCDAENTQLSEAHVEKSESCKTEFASAYRAHTASASAKLRVLYQGNNITVTAYANGDHAVTVKDAKFIVGPMSSAWTPFDNKIVVYKGDVYNMDYPPFGAGRPGQFGDIQSRTPESKDVYANTQLVLQRPAAGTVHVPYSQAPSGFKYWLKERGASLQHTAPFGCQIATNPVRAMNCAVGNMPISIDIPDAAFTRVVDAPSLTDMSCEVPACTHSSDFGGVAIIKYAVSKKGKCAVHSMTNAVTIREAEIEVEGNSQLQISFSTALASAEFRVQVCSTQVHCAAECHPPKDHIVNYPASHTTLGVQDISATAMSWVQKITGGVGLVVAVAALILIVVLCVSFSRH

SEQ ID NO: 11 - protein, 987 aa, Artificial Sequence
  synthetic polypeptide - NP_690589.2 - E3-E2-6K-E1
SLAIPVMCLLANTTFPCSQPPCIPCCYEKEPEETLRMLEDNVMRPGYYQLLQASLTCSPHRQRRSTKDNFNVYKATRPYLAHCPDCGEGHSCHSPVALERIRNEATDGTLKIQVSLQIGIGTDDSHDWTKLRYMDNHIPADAGRAGLFVRTSAPCTITGTMGHFILARCPKGETLTVGFTDSRKISHSCTHPFHHDPPVIGREKFHSRPQHGKELPCSTYVQSNAATAEEIEVHMPPDTPDRTLLSQQSGNVKITVNSQTVRYKCNCGGSNEGLITTDKVINNCKVDQCHAAVTNHKKWQYNSPLVPRNAELGDRKGKIHIPFPLANVTCMVPKARNPTVTYGKNQVIMLLYPDHPTLLSYRSMGEEPNYQEEWVTHKKEVVLTVPTEGLEVTWGNNEPYKYWPQLSANGTAHGHPHEIILYYYELYPTMTVVVVSVASFILLSMVGMAVGMCMCARRRCITPYELTPGATVPFLLSLICCIRTAKAATYQEAAVYLWNEQQPLFWLQALIPLAALIVLCNCLRLLPCCCKTLAFLAVMSIGAHTVSAYEHVTVIPNTVGVPYKTLVNRPGYSPMVLEMELLSVTLEPTLSLDYITCEYKTVIPSPYVKCCGTAECKDKNLPDYSCKVFTGVYPFMWGGAYCFCDAENTQLSEAHVEKSESCKTEFASAYRAHTASASAKLRVLYQGNNITVTAYANGDHAVTVKDAKFIVGPMSSAWTPFDNKIVVYKGDVYNMDYPPFGAGRPGQFGDIQSRTPESKDVYANTQLVLQRPAAGTVHVPYSQAPSGFKYWLKERGASLQHTAPFGCQIATNPVRAMNCAVGNMPISIDIPDAAFTRVVDAPSLTDMSCEVPACTHSSDFGGVAIIKYAVSKKGKCAVHSMTNAVTIREAEIEVEGNSQLQISFSTALASAEFRVQVCSTQVHCAAECHPPKDHIVNYPASHTTLGVQDISATAMSWVQKITGGVGLVVAVAALILIVVLCVSFSRH